European Patent Application EP 4 464 781 A1, published November 20, 2024. Title: 一种抑制PCSK9基因表达的RNAi剂及其应用. Applicant: 石药集团中奇制药技术（石家庄）有限公司. The sequence listing filed with the application follows.

SEQUENCE LISTING (246 sequences)

SEQ ID NO: 1 - DNA, 97 bp, synthetic construct
  source 1..97: mol_type = other DNA
tctgtcctctctgttgcctttttacagccaacttttctagacctgttttgcttttgtaacttgaagatatttattctgggttttgtagcatttttat

SEQ ID NO: 2 - DNA, 23 bp, synthetic construct
  source 1..23: mol_type = other DNA
tggggctgagctttaaaatggtt

SEQ ID NO: 3 - RNA, 21 nt, synthetic construct
  modified_base 1..21: mod_base = OTHER; note = modified as described in table 7
  source 1..21: mol_type = other RNA
tgtcctctctgttgccttttt

SEQ ID NO: 4 - RNA, 23 nt, synthetic construct
  modified_base 1..23: mod_base = OTHER; note = modified as described in table 7
  source 1..23: mol_type = other RNA
aaaaaggcaacagagaggacaga

SEQ ID NO: 5 - RNA, 21 nt, synthetic construct
  modified_base 1..21: mod_base = OTHER; note = modified as described in table 7
  source 1..21: mol_type = other RNA
gtcctctctgttgccttttta

SEQ ID NO: 6 - RNA, 23 nt, synthetic construct
  modified_base 1..23: mod_base = OTHER; note = modified as described in table 7
  source 1..23: mol_type = other RNA
taaaaaggcaacagagaggacag

SEQ ID NO: 7 - RNA, 21 nt, synthetic construct
  modified_base 1..21: mod_base = OTHER; note = modified as described in table 7
  source 1..21: mol_type = other RNA
agacctgttttgcttttgtaa

SEQ ID NO: 8 - RNA, 23 nt, synthetic construct
  modified_base 1..23: mod_base = OTHER; note = modified as described in table 7
  source 1..23: mol_type = other RNA
ttacaaaagcaaaacaggtctag

SEQ ID NO: 9 - RNA, 21 nt, synthetic construct
  modified_base 1..21: mod_base = OTHER; note = modified as described in table 7
  source 1..21: mol_type = other RNA
gacctgttttgcttttgtaac

SEQ ID NO: 10 - RNA, 23 nt, synthetic construct
  modified_base 1..23: mod_base = OTHER; note = modified as described in table 7
  source 1..23: mol_type = other RNA
gttacaaaagcaaaacaggtcta

SEQ ID NO: 11 - RNA, 21 nt, synthetic construct
  modified_base 1..21: mod_base = OTHER; note = modified as described in table 7
  source 1..21: mol_type = other RNA
acctgttttgcttttgtaact

SEQ ID NO: 12 - RNA, 23 nt, synthetic construct
  modified_base 1..23: mod_base = OTHER; note = modified as described in table 7
  source 1..23: mol_type = other RNA
agttacaaaagcaaaacaggtct

SEQ ID NO: 13 - RNA, 21 nt, synthetic construct
  modified_base 1..21: mod_base = OTHER; note = modified as described in table 7
  source 1..21: mol_type = other RNA
ctgttttgcttttgtaacttg

SEQ ID NO: 14 - RNA, 23 nt, synthetic construct
  modified_base 1..23: mod_base = OTHER; note = modified as described in table 7
  source 1..23: mol_type = other RNA
caagttacaaaagcaaaacaggt

SEQ ID NO: 15 - RNA, 21 nt, synthetic construct
  modified_base 1..21: mod_base = OTHER; note = modified as described in table 7
  source 1..21: mol_type = other RNA
tttgtaacttgaagatattta

SEQ ID NO: 16 - RNA, 23 nt, synthetic construct
  modified_base 1..23: mod_base = OTHER; note = modified as described in table 7
  source 1..23: mol_type = other RNA
taaatatcttcaagttacaaaag

SEQ ID NO: 17 - RNA, 21 nt, synthetic construct
  modified_base 1..21: mod_base = OTHER; note = modified as described in table 7
  source 1..21: mol_type = other RNA
ttgtaacttgaagatatttat

SEQ ID NO: 18 - RNA, 23 nt, synthetic construct
  modified_base 1..23: mod_base = OTHER; note = modified as described in table 7
  source 1..23: mol_type = other RNA
ataaatatcttcaagttacaaaa

SEQ ID NO: 19 - RNA, 21 nt, synthetic construct
  modified_base 1..21: mod_base = OTHER; note = modified as described in table 7
  source 1..21: mol_type = other RNA
tgtaacttgaagatatttatt

SEQ ID NO: 20 - RNA, 23 nt, synthetic construct
  modified_base 1..23: mod_base = OTHER; note = modified as described in table 7
  source 1..23: mol_type = other RNA
aataaatatcttcaagttacaaa

SEQ ID NO: 21 - RNA, 21 nt, synthetic construct
  modified_base 1..21: mod_base = OTHER; note = modified as described in table 7
  source 1..21: mol_type = other RNA
gtaacttgaagatatttattc

SEQ ID NO: 22 - RNA, 23 nt, synthetic construct
  modified_base 1..23: mod_base = OTHER; note = modified as described in table 7
  source 1..23: mol_type = other RNA
gaataaatatcttcaagttacaa

SEQ ID NO: 23 - RNA, 21 nt, synthetic construct
  modified_base 1..21: mod_base = OTHER; note = modified as described in table 7
  source 1..21: mol_type = other RNA
atatttattctgggttttgta

SEQ ID NO: 24 - RNA, 23 nt, synthetic construct
  modified_base 1..23: mod_base = OTHER; note = modified as described in table 7
  source 1..23: mol_type = other RNA
tacaaaacccagaataaatatct

SEQ ID NO: 25 - RNA, 21 nt, synthetic construct
  modified_base 1..21: mod_base = OTHER; note = modified as described in table 7
  source 1..21: mol_type = other RNA
tttattctgggttttgtagca

SEQ ID NO: 26 - RNA, 23 nt, synthetic construct
  modified_base 1..23: mod_base = OTHER; note = modified as described in table 7
  source 1..23: mol_type = other RNA
tgctacaaaacccagaataaata

SEQ ID NO: 27 - RNA, 21 nt, synthetic construct
  modified_base 1..21: mod_base = OTHER; note = modified as described in table 7
  source 1..21: mol_type = other RNA
attctgggttttgtagcattt

SEQ ID NO: 28 - RNA, 23 nt, synthetic construct
  modified_base 1..23: mod_base = OTHER; note = modified as described in table 7
  source 1..23: mol_type = other RNA
aaatgctacaaaacccagaataa

SEQ ID NO: 29 - RNA, 21 nt, synthetic construct
  modified_base 1..21: mod_base = OTHER; note = modified as described in table 7
  source 1..21: mol_type = other RNA
ctgggttttgtagcattttta

SEQ ID NO: 30 - RNA, 23 nt, synthetic construct
  modified_base 1..23: mod_base = OTHER; note = modified as described in table 7
  source 1..23: mol_type = other RNA
taaaaatgctacaaaacccagaa

SEQ ID NO: 31 - RNA, 21 nt, synthetic construct
  modified_base 1..21: mod_base = OTHER; note = modified as described in table 7
  source 1..21: mol_type = other RNA
tgggttttgtagcatttttat

SEQ ID NO: 32 - RNA, 23 nt, synthetic construct
  modified_base 1..23: mod_base = OTHER; note = modified as described in table 7
  source 1..23: mol_type = other RNA
ataaaaatgctacaaaacccaga

SEQ ID NO: 33 - RNA, 21 nt, synthetic construct
  modified_base 1..21: mod_base = OTHER; note = modified as described in table 7
  source 1..21: mol_type = other RNA
gggctgagctttaaaatggtt

SEQ ID NO: 34 - RNA, 23 nt, synthetic construct
  modified_base 1..23: mod_base = OTHER; note = modified as described in table 7
  source 1..23: mol_type = other RNA
aaccattttaaagctcagcccca

SEQ ID NO: 35 - RNA, 21 nt, synthetic construct
  modified_base 1..21: mod_base = OTHER; note = modified as described in table 8
  source 1..21: mol_type = other RNA
agacctgttttgcttttgtaa

SEQ ID NO: 36 - RNA, 21 nt, synthetic construct
  modified_base 1..21: mod_base = OTHER; note = modified as described in table 8
  source 1..21: mol_type = other RNA
agacctgttttgcttttgtaa

SEQ ID NO: 37 - RNA, 21 nt, synthetic construct
  modified_base 1..21: mod_base = OTHER; note = modified as described in table 8
  source 1..21: mol_type = other RNA
agacctgttttgcttttgtaa

SEQ ID NO: 38 - RNA, 21 nt, synthetic construct
  modified_base 1..21: mod_base = OTHER; note = modified as described in table 8
  source 1..21: mol_type = other RNA
agacctgttttgcttttgtaa

SEQ ID NO: 39 - RNA, 21 nt, synthetic construct
  modified_base 1..21: mod_base = OTHER; note = modified as described in table 8
  source 1..21: mol_type = other RNA
agacctgttttgcttttgtaa

SEQ ID NO: 40 - DNA, 35 bp, synthetic construct
  misc_feature 28..29: note = DNA
  source 1..35: mol_type = other DNA
  modified_base 1..35: mod_base = OTHER; note = modified as described in table 8
agacctgttttgcttttgtaagcagccgaggctgc

SEQ ID NO: 41 - RNA, 23 nt, synthetic construct
  modified_base 1..23: mod_base = OTHER; note = modified as described in table 12
  source 1..23: mol_type = other RNA
ttacaaaagcaaaacaggtctag

SEQ ID NO: 42 - RNA, 21 nt, synthetic construct
  modified_base 1..21: mod_base = OTHER; note = modified as described in table 12
  source 1..21: mol_type = other RNA
agacctgttttgcttttgtaa

SEQ ID NO: 43 - RNA, 23 nt, synthetic construct
  modified_base 1..23: mod_base = OTHER; note = modified as described in table 12
  source 1..23: mol_type = other RNA
ttacaaaagcaaaacaggtctag

SEQ ID NO: 44 - RNA, 21 nt, synthetic construct
  modified_base 1..21: mod_base = OTHER; note = modified as described in table 12
  source 1..21: mol_type = other RNA
agacctgttttgcttttgtaa

SEQ ID NO: 45 - RNA, 23 nt, synthetic construct
  modified_base 1..23: mod_base = OTHER; note = modified as described in table 12
  source 1..23: mol_type = other RNA
ttacaaaagcaaaacaggtctag

SEQ ID NO: 46 - DNA, 21 bp, synthetic construct
  misc_feature 11: note = DNA
  source 1..21: mol_type = other DNA
  modified_base 1..21: mod_base = OTHER; note = modified as described in table 12
agacctgttttgcttttgtaa

SEQ ID NO: 47 - RNA, 23 nt, synthetic construct
  modified_base 1..23: mod_base = OTHER; note = modified as described in table 12
  source 1..23: mol_type = other RNA
caagttacaaaagcaaaacaggt

SEQ ID NO: 48 - RNA, 21 nt, synthetic construct
  modified_base 1..21: mod_base = OTHER; note = modified as described in table 12
  source 1..21: mol_type = other RNA
ctgttttgcttttgtaacttg

SEQ ID NO: 49 - RNA, 23 nt, synthetic construct
  modified_base 1..23: mod_base = OTHER; note = modified as described in table 12
  source 1..23: mol_type = other RNA
caagttacaaaagcaaaacaggt

SEQ ID NO: 50 - RNA, 21 nt, synthetic construct
  modified_base 1..21: mod_base = OTHER; note = modified as described in table 12
  source 1..21: mol_type = other RNA
ctgttttgcttttgtaacttg

SEQ ID NO: 51 - RNA, 23 nt, synthetic construct
  modified_base 1..23: mod_base = OTHER; note = modified as described in table 12
  source 1..23: mol_type = other RNA
caagttacaaaagcaaaacaggt

SEQ ID NO: 52 - DNA, 21 bp, synthetic construct
  misc_feature 11: note = DNA
  source 1..21: mol_type = other DNA
  modified_base 1..21: mod_base = OTHER; note = modified as described in table 12
ctgttttgcttttgtaacttg

SEQ ID NO: 53 - RNA, 21 nt, synthetic construct
  modified_base 1..21: mod_base = OTHER; note = modified as described in table 12
  source 1..21: mol_type = other RNA
ctgttttgcttttgtaacttg

SEQ ID NO: 54 - RNA, 23 nt, synthetic construct
  modified_base 1..23: mod_base = OTHER; note = modified as described in table 12
  source 1..23: mol_type = other RNA
caagttacaaaagcaaaacaggt

SEQ ID NO: 55 - RNA, 23 nt, synthetic construct
  modified_base 1..23: mod_base = OTHER; note = modified as described in table 12
  source 1..23: mol_type = other RNA
caagttacaaaagcaaaacaggt

SEQ ID NO: 56 - RNA, 23 nt, synthetic construct
  modified_base 1..23: mod_base = OTHER; note = modified as described in table 12
  source 1..23: mol_type = other RNA
caagttacaaaagcaaaacaggt

SEQ ID NO: 57 - RNA, 21 nt, synthetic construct
  source 1..21: mol_type = other RNA
ctagacctgttttgcttttgt

SEQ ID NO: 58 - RNA, 23 nt, synthetic construct
  source 1..23: mol_type = other RNA
acaaaagcaaaacaggtctagaa

SEQ ID NO: 59 - RNA, 21 nt, synthetic construct
  source 1..21: mol_type = other RNA
ctggggctgagctttaaaatg

SEQ ID NO: 60 - RNA, 23 nt, synthetic construct
  source 1..23: mol_type = other RNA
cattttaaagctcagccccagcc

SEQ ID NO: 61 - RNA, 21 nt, synthetic construct
  source 1..21: mol_type = other RNA
gggctgagctttaaaatggtt

SEQ ID NO: 62 - RNA, 23 nt, synthetic construct
  source 1..23: mol_type = other RNA
aaccattttaaagctcagcccca

SEQ ID NO: 63 - RNA, 21 nt, synthetic construct
  source 1..21: mol_type = other RNA
gctgagctttaaaatggttcc

SEQ ID NO: 64 - RNA, 23 nt, synthetic construct
  source 1..23: mol_type = other RNA
ggaaccattttaaagctcagccc

SEQ ID NO: 65 - RNA, 21 nt, synthetic construct
  source 1..21: mol_type = other RNA
cctggcccttgagtggggcag

SEQ ID NO: 66 - RNA, 23 nt, synthetic construct
  source 1..23: mol_type = other RNA
ctgccccactcaagggccaggcc

SEQ ID NO: 67 - RNA, 21 nt, synthetic construct
  source 1..21: mol_type = other RNA
ggaggtgccaggaagctccct

SEQ ID NO: 68 - RNA, 23 nt, synthetic construct
  source 1..23: mol_type = other RNA
agggagcttcctggcacctccac

SEQ ID NO: 69 - RNA, 21 nt, synthetic construct
  source 1..21: mol_type = other RNA
gaggtgccaggaagctccctc

SEQ ID NO: 70 - RNA, 23 nt, synthetic construct
  source 1..23: mol_type = other RNA
gagggagcttcctggcacctcca

SEQ ID NO: 71 - RNA, 21 nt, synthetic construct
  source 1..21: mol_type = other RNA
cctcactgtggggcatttcac

SEQ ID NO: 72 - RNA, 23 nt, synthetic construct
  source 1..23: mol_type = other RNA
gtgaaatgccccacagtgaggga

SEQ ID NO: 73 - RNA, 21 nt, synthetic construct
  source 1..21: mol_type = other RNA
ctcactgtggggcatttcacc

SEQ ID NO: 74 - RNA, 23 nt, synthetic construct
  source 1..23: mol_type = other RNA
ggtgaaatgccccacagtgaggg

SEQ ID NO: 75 - RNA, 21 nt, synthetic construct
  source 1..21: mol_type = other RNA
tgtggggcatttcaccattca

SEQ ID NO: 76 - RNA, 23 nt, synthetic construct
  source 1..23: mol_type = other RNA
tgaatggtgaaatgccccacagt

SEQ ID NO: 77 - RNA, 21 nt, synthetic construct
  source 1..21: mol_type = other RNA
acttttattgagctcttgttc

SEQ ID NO: 78 - RNA, 23 nt, synthetic construct
  source 1..23: mol_type = other RNA
gaacaagagctcaataaaagtca

SEQ ID NO: 79 - RNA, 21 nt, synthetic construct
  source 1..21: mol_type = other RNA
ggcatctagccagaggctgga

SEQ ID NO: 80 - RNA, 23 nt, synthetic construct
  source 1..23: mol_type = other RNA
tccagcctctggctagatgccat

SEQ ID NO: 81 - RNA, 21 nt, synthetic construct
  source 1..21: mol_type = other RNA
gcatctagccagaggctggag

SEQ ID NO: 82 - RNA, 23 nt, synthetic construct
  source 1..23: mol_type = other RNA
ctccagcctctggctagatgcca

SEQ ID NO: 83 - RNA, 21 nt, synthetic construct
  source 1..21: mol_type = other RNA
ggtaacagtgaggctgggaag

SEQ ID NO: 84 - RNA, 23 nt, synthetic construct
  source 1..23: mol_type = other RNA
cttcccagcctcactgttacccg

SEQ ID NO: 85 - RNA, 21 nt, synthetic construct
  source 1..21: mol_type = other RNA
aggctgggaaggggaacacag

SEQ ID NO: 86 - RNA, 23 nt, synthetic construct
  source 1..23: mol_type = other RNA
ctgtgttccccttcccagcctca

SEQ ID NO: 87 - RNA, 21 nt, synthetic construct
  source 1..21: mol_type = other RNA
ggaaggggaacacagaccagg

SEQ ID NO: 88 - RNA, 23 nt, synthetic construct
  source 1..23: mol_type = other RNA
cctggtctgtgttccccttccca

SEQ ID NO: 89 - RNA, 21 nt, synthetic construct
  source 1..21: mol_type = other RNA
aggggaacacagaccaggaag

SEQ ID NO: 90 - RNA, 23 nt, synthetic construct
  source 1..23: mol_type = other RNA
cttcctggtctgtgttccccttc

SEQ ID NO: 91 - RNA, 21 nt, synthetic construct
  source 1..21: mol_type = other RNA
ggggaacacagaccaggaagc

SEQ ID NO: 92 - RNA, 23 nt, synthetic construct
  source 1..23: mol_type = other RNA
gcttcctggtctgtgttcccctt

SEQ ID NO: 93 - RNA, 21 nt, synthetic construct
  source 1..21: mol_type = other RNA
gggaacacagaccaggaagct

SEQ ID NO: 94 - RNA, 23 nt, synthetic construct
  source 1..23: mol_type = other RNA
agcttcctggtctgtgttcccct

SEQ ID NO: 95 - RNA, 21 nt, synthetic construct
  source 1..21: mol_type = other RNA
ggaacacagaccaggaagctc

SEQ ID NO: 96 - RNA, 23 nt, synthetic construct
  source 1..23: mol_type = other RNA
gagcttcctggtctgtgttcccc

SEQ ID NO: 97 - RNA, 21 nt, synthetic construct
  source 1..21: mol_type = other RNA
acccaagcaagcagacattta

SEQ ID NO: 98 - RNA, 23 nt, synthetic construct
  source 1..23: mol_type = other RNA
taaatgtctgcttgcttgggtgg

SEQ ID NO: 99 - RNA, 21 nt, synthetic construct
  source 1..21: mol_type = other RNA
cccaagcaagcagacatttat

SEQ ID NO: 100 - RNA, 23 nt, synthetic construct
  source 1..23: mol_type = other RNA
ataaatgtctgcttgcttgggtg

SEQ ID NO: 101 - RNA, 21 nt, synthetic construct
  source 1..21: mol_type = other RNA
ccaagcaagcagacatttatc

SEQ ID NO: 102 - RNA, 23 nt, synthetic construct
  source 1..23: mol_type = other RNA
gataaatgtctgcttgcttgggt

SEQ ID NO: 103 - RNA, 21 nt, synthetic construct
  source 1..21: mol_type = other RNA
caagcaagcagacatttatct

SEQ ID NO: 104 - RNA, 23 nt, synthetic construct
  source 1..23: mol_type = other RNA
agataaatgtctgcttgcttggg

SEQ ID NO: 105 - RNA, 21 nt, synthetic construct
  source 1..21: mol_type = other RNA
gcagacatttatcttttgggt

SEQ ID NO: 106 - RNA, 23 nt, synthetic construct
  source 1..23: mol_type = other RNA
acccaaaagataaatgtctgctt

SEQ ID NO: 107 - RNA, 21 nt, synthetic construct
  source 1..21: mol_type = other RNA
tttgggtctgtcctctctgtt

SEQ ID NO: 108 - RNA, 23 nt, synthetic construct
  source 1..23: mol_type = other RNA
aacagagaggacagacccaaaag

SEQ ID NO: 109 - RNA, 21 nt, synthetic construct
  source 1..21: mol_type = other RNA
tgggtctgtcctctctgttgc

SEQ ID NO: 110 - RNA, 23 nt, synthetic construct
  source 1..23: mol_type = other RNA
gcaacagagaggacagacccaaa

SEQ ID NO: 111 - RNA, 21 nt, synthetic construct
  source 1..21: mol_type = other RNA
gggtctgtcctctctgttgcc

SEQ ID NO: 112 - RNA, 23 nt, synthetic construct
  source 1..23: mol_type = other RNA
ggcaacagagaggacagacccaa

SEQ ID NO: 113 - RNA, 21 nt, synthetic construct
  source 1..21: mol_type = other RNA
ggtctgtcctctctgttgcct

SEQ ID NO: 114 - RNA, 23 nt, synthetic construct
  source 1..23: mol_type = other RNA
aggcaacagagaggacagaccca

SEQ ID NO: 115 - RNA, 21 nt, synthetic construct
  source 1..21: mol_type = other RNA
gtctgtcctctctgttgcctt

SEQ ID NO: 116 - RNA, 23 nt, synthetic construct
  source 1..23: mol_type = other RNA
aaggcaacagagaggacagaccc

SEQ ID NO: 117 - RNA, 21 nt, synthetic construct
  source 1..21: mol_type = other RNA
ctgtcctctctgttgcctttt

SEQ ID NO: 118 - RNA, 23 nt, synthetic construct
  source 1..23: mol_type = other RNA
aaaaggcaacagagaggacagac

SEQ ID NO: 119 - RNA, 21 nt, synthetic construct
  source 1..21: mol_type = other RNA
tgtcctctctgttgccttttt

SEQ ID NO: 120 - RNA, 23 nt, synthetic construct
  source 1..23: mol_type = other RNA
aaaaaggcaacagagaggacaga

SEQ ID NO: 121 - RNA, 21 nt, synthetic construct
  source 1..21: mol_type = other RNA
gtcctctctgttgccttttta

SEQ ID NO: 122 - RNA, 23 nt, synthetic construct
  source 1..23: mol_type = other RNA
taaaaaggcaacagagaggacag

SEQ ID NO: 123 - RNA, 21 nt, synthetic construct
  source 1..21: mol_type = other RNA
tcctctctgttgcctttttac

SEQ ID NO: 124 - RNA, 23 nt, synthetic construct
  source 1..23: mol_type = other RNA
gtaaaaaggcaacagagaggaca

SEQ ID NO: 125 - RNA, 21 nt, synthetic construct
  source 1..21: mol_type = other RNA
cctctctgttgcctttttaca

SEQ ID NO: 126 - RNA, 23 nt, synthetic construct
  source 1..23: mol_type = other RNA
tgtaaaaaggcaacagagaggac

SEQ ID NO: 127 - RNA, 21 nt, synthetic construct
  source 1..21: mol_type = other RNA
ctctgttgcctttttacagcc

SEQ ID NO: 128 - RNA, 23 nt, synthetic construct
  source 1..23: mol_type = other RNA
ggctgtaaaaaggcaacagagag

SEQ ID NO: 129 - RNA, 21 nt, synthetic construct
  source 1..21: mol_type = other RNA
tctgttgcctttttacagcca

SEQ ID NO: 130 - RNA, 23 nt, synthetic construct
  source 1..23: mol_type = other RNA
tggctgtaaaaaggcaacagaga

SEQ ID NO: 131 - RNA, 21 nt, synthetic construct
  source 1..21: mol_type = other RNA
ttgcctttttacagccaactt

SEQ ID NO: 132 - RNA, 23 nt, synthetic construct
  source 1..23: mol_type = other RNA
aagttggctgtaaaaaggcaaca

SEQ ID NO: 133 - RNA, 21 nt, synthetic construct
  source 1..21: mol_type = other RNA
agacctgttttgcttttgtaa

SEQ ID NO: 134 - RNA, 23 nt, synthetic construct
  source 1..23: mol_type = other RNA
ttacaaaagcaaaacaggtctag

SEQ ID NO: 135 - RNA, 21 nt, synthetic construct
  source 1..21: mol_type = other RNA
gacctgttttgcttttgtaac

SEQ ID NO: 136 - RNA, 23 nt, synthetic construct
  source 1..23: mol_type = other RNA
gttacaaaagcaaaacaggtcta

SEQ ID NO: 137 - RNA, 21 nt, synthetic construct
  source 1..21: mol_type = other RNA
acctgttttgcttttgtaact

SEQ ID NO: 138 - RNA, 23 nt, synthetic construct
  source 1..23: mol_type = other RNA
agttacaaaagcaaaacaggtct

SEQ ID NO: 139 - RNA, 21 nt, synthetic construct
  source 1..21: mol_type = other RNA
ctgttttgcttttgtaacttg

SEQ ID NO: 140 - RNA, 23 nt, synthetic construct
  source 1..23: mol_type = other RNA
caagttacaaaagcaaaacaggt

SEQ ID NO: 141 - RNA, 21 nt, synthetic construct
  source 1..21: mol_type = other RNA
tgttttgcttttgtaacttga

SEQ ID NO: 142 - RNA, 23 nt, synthetic construct
  source 1..23: mol_type = other RNA
tcaagttacaaaagcaaaacagg

SEQ ID NO: 143 - RNA, 21 nt, synthetic construct
  source 1..21: mol_type = other RNA
tttgtaacttgaagatattta

SEQ ID NO: 144 - RNA, 23 nt, synthetic construct
  source 1..23: mol_type = other RNA
taaatatcttcaagttacaaaag

SEQ ID NO: 145 - RNA, 21 nt, synthetic construct
  source 1..21: mol_type = other RNA
ttgtaacttgaagatatttat

SEQ ID NO: 146 - RNA, 23 nt, synthetic construct
  source 1..23: mol_type = other RNA
ataaatatcttcaagttacaaaa

SEQ ID NO: 147 - RNA, 21 nt, synthetic construct
  source 1..21: mol_type = other RNA
tgtaacttgaagatatttatt

SEQ ID NO: 148 - RNA, 23 nt, synthetic construct
  source 1..23: mol_type = other RNA
aataaatatcttcaagttacaaa

SEQ ID NO: 149 - RNA, 21 nt, synthetic construct
  source 1..21: mol_type = other RNA
gtaacttgaagatatttattc

SEQ ID NO: 150 - RNA, 23 nt, synthetic construct
  source 1..23: mol_type = other RNA
gaataaatatcttcaagttacaa

SEQ ID NO: 151 - RNA, 21 nt, synthetic construct
  source 1..21: mol_type = other RNA
atatttattctgggttttgta

SEQ ID NO: 152 - RNA, 23 nt, synthetic construct
  source 1..23: mol_type = other RNA
tacaaaacccagaataaatatct

SEQ ID NO: 153 - RNA, 21 nt, synthetic construct
  source 1..21: mol_type = other RNA
tatttattctgggttttgtag

SEQ ID NO: 154 - RNA, 23 nt, synthetic construct
  source 1..23: mol_type = other RNA
ctacaaaacccagaataaatatc

SEQ ID NO: 155 - RNA, 21 nt, synthetic construct
  source 1..21: mol_type = other RNA
tttattctgggttttgtagca

SEQ ID NO: 156 - RNA, 23 nt, synthetic construct
  source 1..23: mol_type = other RNA
tgctacaaaacccagaataaata

SEQ ID NO: 157 - RNA, 21 nt, synthetic construct
  source 1..21: mol_type = other RNA
attctgggttttgtagcattt

SEQ ID NO: 158 - RNA, 23 nt, synthetic construct
  source 1..23: mol_type = other RNA
aaatgctacaaaacccagaataa

SEQ ID NO: 159 - RNA, 21 nt, synthetic construct
  source 1..21: mol_type = other RNA
ctgggttttgtagcattttta

SEQ ID NO: 160 - RNA, 23 nt, synthetic construct
  source 1..23: mol_type = other RNA
taaaaatgctacaaaacccagaa

SEQ ID NO: 161 - RNA, 21 nt, synthetic construct
  source 1..21: mol_type = other RNA
tgggttttgtagcatttttat

SEQ ID NO: 162 - RNA, 23 nt, synthetic construct
  source 1..23: mol_type = other RNA
ataaaaatgctacaaaacccaga

SEQ ID NO: 163 - RNA, 21 nt, synthetic construct
  source 1..21: mol_type = other RNA
cccgccggggatacctcacca

SEQ ID NO: 164 - RNA, 21 nt, synthetic construct
  source 1..21: mol_type = other RNA
gtgaggtatccccggcgggca

SEQ ID NO: 165 - RNA, 21 nt, synthetic construct
  source 1..21: mol_type = other RNA
ggggatacctcaccaagatcc

SEQ ID NO: 166 - RNA, 21 nt, synthetic construct
  source 1..21: mol_type = other RNA
atcttggtgaggtatccccgg

SEQ ID NO: 167 - RNA, 21 nt, synthetic construct
  source 1..21: mol_type = other RNA
gggatacctcaccaagatcct

SEQ ID NO: 168 - RNA, 21 nt, synthetic construct
  source 1..21: mol_type = other RNA
gatcttggtgaggtatccccg

SEQ ID NO: 169 - RNA, 21 nt, synthetic construct
  source 1..21: mol_type = other RNA
accaagatcctgcatgtcttc

SEQ ID NO: 170 - RNA, 21 nt, synthetic construct
  source 1..21: mol_type = other RNA
agacatgcaggatcttggtga

SEQ ID NO: 171 - RNA, 21 nt, synthetic construct
  source 1..21: mol_type = other RNA
cccatgtcgactacatcgagg

SEQ ID NO: 172 - RNA, 21 nt, synthetic construct
  source 1..21: mol_type = other RNA
tcgatgtagtcgacatggggc

SEQ ID NO: 173 - RNA, 21 nt, synthetic construct
  source 1..21: mol_type = other RNA
ccaactttggccgctgtgtgg

SEQ ID NO: 174 - RNA, 21 nt, synthetic construct
  source 1..21: mol_type = other RNA
acacagcggccaaagttggtc

SEQ ID NO: 175 - RNA, 21 nt, synthetic construct
  source 1..21: mol_type = other RNA
cgctgtgtggacctctttgcc

SEQ ID NO: 176 - RNA, 21 nt, synthetic construct
  source 1..21: mol_type = other RNA
caaagaggtccacacagcggc

SEQ ID NO: 177 - RNA, 21 nt, synthetic construct
  source 1..21: mol_type = other RNA
cacaacgcttttgggggtgag

SEQ ID NO: 178 - RNA, 21 nt, synthetic construct
  source 1..21: mol_type = other RNA
cacccccaaaagcgttgtggg

SEQ ID NO: 179 - RNA, 21 nt, synthetic construct
  source 1..21: mol_type = other RNA
acaacgcttttgggggtgagg

SEQ ID NO: 180 - RNA, 21 nt, synthetic construct
  source 1..21: mol_type = other RNA
tcacccccaaaagcgttgtgg

SEQ ID NO: 181 - RNA, 21 nt, synthetic construct
  source 1..21: mol_type = other RNA
caacgcttttgggggtgaggg

SEQ ID NO: 182 - RNA, 21 nt, synthetic construct
  source 1..21: mol_type = other RNA
ctcacccccaaaagcgttgtg

SEQ ID NO: 183 - RNA, 21 nt, synthetic construct
  source 1..21: mol_type = other RNA
gtgagggtgtctacgccattg

SEQ ID NO: 184 - RNA, 21 nt, synthetic construct
  source 1..21: mol_type = other RNA
atggcgtagacaccctcaccc

SEQ ID NO: 185 - RNA, 21 nt, synthetic construct
  source 1..21: mol_type = other RNA
tgagggtgtctacgccattgc

SEQ ID NO: 186 - RNA, 21 nt, synthetic construct
  source 1..21: mol_type = other RNA
aatggcgtagacaccctcacc

SEQ ID NO: 187 - RNA, 21 nt, synthetic construct
  source 1..21: mol_type = other RNA
gagggtgtctacgccattgcc

SEQ ID NO: 188 - RNA, 21 nt, synthetic construct
  source 1..21: mol_type = other RNA
caatggcgtagacaccctcac

SEQ ID NO: 189 - RNA, 21 nt, synthetic construct
  source 1..21: mol_type = other RNA
gggtgtctacgccattgccag

SEQ ID NO: 190 - RNA, 21 nt, synthetic construct
  source 1..21: mol_type = other RNA
ggcaatggcgtagacaccctc

SEQ ID NO: 191 - RNA, 21 nt, synthetic construct
  source 1..21: mol_type = other RNA
ggtgtctacgccattgccagg

SEQ ID NO: 192 - RNA, 21 nt, synthetic construct
  source 1..21: mol_type = other RNA
tggcaatggcgtagacaccct

SEQ ID NO: 193 - RNA, 21 nt, synthetic construct
  source 1..21: mol_type = other RNA
gtgtctacgccattgccaggt

SEQ ID NO: 194 - RNA, 21 nt, synthetic construct
  source 1..21: mol_type = other RNA
ctggcaatggcgtagacaccc

SEQ ID NO: 195 - RNA, 21 nt, synthetic construct
  source 1..21: mol_type = other RNA
tgtctacgccattgccaggtg

SEQ ID NO: 196 - RNA, 21 nt, synthetic construct
  source 1..21: mol_type = other RNA
cctggcaatggcgtagacacc

SEQ ID NO: 197 - RNA, 21 nt, synthetic construct
  source 1..21: mol_type = other RNA
ctacgccattgccaggtgctg

SEQ ID NO: 198 - RNA, 21 nt, synthetic construct
  source 1..21: mol_type = other RNA
gcacctggcaatggcgtagac

SEQ ID NO: 199 - RNA, 21 nt, synthetic construct
  source 1..21: mol_type = other RNA
tacgccattgccaggtgctgc

SEQ ID NO: 200 - RNA, 21 nt, synthetic construct
  source 1..21: mol_type = other RNA
agcacctggcaatggcgtaga

SEQ ID NO: 201 - RNA, 21 nt, synthetic construct
  source 1..21: mol_type = other RNA
cacccacaagccgcctgtgct

SEQ ID NO: 202 - RNA, 21 nt, synthetic construct
  source 1..21: mol_type = other RNA
cacaggcggcttgtgggtgcc

SEQ ID NO: 203 - RNA, 21 nt, synthetic construct
  source 1..21: mol_type = other RNA
cccacaagccgcctgtgctga

SEQ ID NO: 204 - RNA, 21 nt, synthetic construct
  source 1..21: mol_type = other RNA
agcacaggcggcttgtgggtg

SEQ ID NO: 205 - RNA, 21 nt, synthetic construct
  source 1..21: mol_type = other RNA
ccacaagccgcctgtgctgag

SEQ ID NO: 206 - RNA, 21 nt, synthetic construct
  source 1..21: mol_type = other RNA
cagcacaggcggcttgtgggt

SEQ ID NO: 207 - RNA, 21 nt, synthetic construct
  source 1..21: mol_type = other RNA
cacgaggtcagcccaaccagt

SEQ ID NO: 208 - RNA, 21 nt, synthetic construct
  source 1..21: mol_type = other RNA
tggttgggctgacctcgtggc

SEQ ID NO: 209 - RNA, 21 nt, synthetic construct
  source 1..21: mol_type = other RNA
cgaggtcagcccaaccagtgc

SEQ ID NO: 210 - RNA, 21 nt, synthetic construct
  source 1..21: mol_type = other RNA
actggttgggctgacctcgtg

SEQ ID NO: 211 - RNA, 21 nt, synthetic construct
  source 1..21: mol_type = other RNA
gaggtcagcccaaccagtgcg

SEQ ID NO: 212 - RNA, 21 nt, synthetic construct
  source 1..21: mol_type = other RNA
cactggttgggctgacctcgt

SEQ ID NO: 213 - RNA, 21 nt, synthetic construct
  source 1..21: mol_type = other RNA
gtcaggagccgggacgtcagc

SEQ ID NO: 214 - RNA, 21 nt, synthetic construct
  source 1..21: mol_type = other RNA
tgacgtcccggctcctgacta

SEQ ID NO: 215 - RNA, 21 nt, synthetic construct
  source 1..21: mol_type = other RNA
cggcaccctcataggcctgga

SEQ ID NO: 216 - RNA, 23 nt, synthetic construct
  source 1..23: mol_type = other RNA
tccaggcctatgagggtgccgct

SEQ ID NO: 217 - RNA, 21 nt, synthetic construct
  source 1..21: mol_type = other RNA
gcaccctcataggcctggagt

SEQ ID NO: 218 - RNA, 23 nt, synthetic construct
  source 1..23: mol_type = other RNA
actccaggcctatgagggtgccg

SEQ ID NO: 219 - RNA, 21 nt, synthetic construct
  source 1..21: mol_type = other RNA
accctcataggcctggagttt

SEQ ID NO: 220 - RNA, 23 nt, synthetic construct
  source 1..23: mol_type = other RNA
aaactccaggcctatgagggtgc

SEQ ID NO: 221 - RNA, 21 nt, synthetic construct
  source 1..21: mol_type = other RNA
cctcataggcctggagtttat

SEQ ID NO: 222 - RNA, 23 nt, synthetic construct
  source 1..23: mol_type = other RNA
ataaactccaggcctatgagggt

SEQ ID NO: 223 - RNA, 21 nt, synthetic construct
  source 1..21: mol_type = other RNA
tcataggcctggagtttattc

SEQ ID NO: 224 - RNA, 23 nt, synthetic construct
  source 1..23: mol_type = other RNA
gaataaactccaggcctatgagg

SEQ ID NO: 225 - RNA, 21 nt, synthetic construct
  source 1..21: mol_type = other RNA
ataggcctggagtttattcgg

SEQ ID NO: 226 - RNA, 23 nt, synthetic construct
  source 1..23: mol_type = other RNA
ccgaataaactccaggcctatga

SEQ ID NO: 227 - RNA, 21 nt, synthetic construct
  source 1..21: mol_type = other RNA
aggcctggagtttattcggaa

SEQ ID NO: 228 - RNA, 23 nt, synthetic construct
  source 1..23: mol_type = other RNA
ttccgaataaactccaggcctat

SEQ ID NO: 229 - RNA, 21 nt, synthetic construct
  source 1..21: mol_type = other RNA
acaggctgctgcccacgtggc

SEQ ID NO: 230 - RNA, 23 nt, synthetic construct
  source 1..23: mol_type = other RNA
gccacgtgggcagcagcctgtga

SEQ ID NO: 231 - RNA, 21 nt, synthetic construct
  source 1..21: mol_type = other RNA
ctgacccccaacctggtggcc

SEQ ID NO: 232 - RNA, 23 nt, synthetic construct
  source 1..23: mol_type = other RNA
ggccaccaggttgggggtcagta

SEQ ID NO: 233 - RNA, 21 nt, synthetic construct
  source 1..21: mol_type = other RNA
ggagctgctgagctgctccag

SEQ ID NO: 234 - RNA, 23 nt, synthetic construct
  source 1..23: mol_type = other RNA
ctggagcagctcagcagctcctc

SEQ ID NO: 235 - RNA, 21 nt, synthetic construct
  source 1..21: mol_type = other RNA
ttcctgctgccatgccccagg

SEQ ID NO: 236 - RNA, 23 nt, synthetic construct
  source 1..23: mol_type = other RNA
cctggggcatggcagcaggaagc

SEQ ID NO: 237 - RNA, 21 nt, synthetic construct
  source 1..21: mol_type = other RNA
ccatctgctgccggagccggc

SEQ ID NO: 238 - RNA, 23 nt, synthetic construct
  source 1..23: mol_type = other RNA
gccggctccggcagcagatggca

SEQ ID NO: 239 - DNA, 19 bp, synthetic construct
  source 1..19: mol_type = other DNA
tgccgacaggatgcagaag

SEQ ID NO: 240 - DNA, 20 bp, synthetic construct
  source 1..20: mol_type = other DNA
gccgatccacacggagtact

SEQ ID NO: 241 - DNA, 27 bp, synthetic construct
  source 1..27: mol_type = other DNA
atcaagatcattgctcctcctgagcgc

SEQ ID NO: 242 - DNA, 18 bp, synthetic construct
  source 1..18: mol_type = other DNA
gatcctgcatgtcttcca

SEQ ID NO: 243 - DNA, 18 bp, synthetic construct
  source 1..18: mol_type = other DNA
gtcctcctcgatgtagtc

SEQ ID NO: 244 - DNA, 21 bp, synthetic construct
  source 1..21: mol_type = other DNA
ccttcttcctggcttcctggt

SEQ ID NO: 245 - DNA, 21 bp, synthetic construct
  misc_feature 11: note = DNA
  source 1..21: mol_type = other DNA
  modified_base 1..21: mod_base = OTHER; note = modified as described in table 12
ctagacctgttttgcttttgt

SEQ ID NO: 246 - RNA, 23 nt, synthetic construct
  modified_base 1..23: mod_base = OTHER; note = modified as described in table 12
  source 1..23: mol_type = other RNA
acaaaagcaaaacaggtctagaa